European Patent Specification EP 3 344 659 B1, published March 26, 2025. Title: MOLECULAR CONSTRUCTS FOR INHIBITING THE FORMATION OF BLOOD CLOT AND/OR TREATING THROMBOSIS. Applicant: Immunwork Inc. The sequence listing filed with the application follows.

SEQUENCE LISTING (35 sequences)

SEQ ID NO: 1 - protein, 4 aa, Artificial Sequence
  filler sequence-1
GGGS

SEQ ID NO: 2 - protein, 4 aa, Artificial Sequence
  filler sequence-2
GSGS

SEQ ID NO: 3 - protein, 4 aa, Artificial Sequence
  filler sequence-3
GGSG

SEQ ID NO: 4 - protein, 5 aa, Artificial Sequence
  filler sequence-4
GSGGS

SEQ ID NO: 5 - protein, 5 aa, Artificial Sequence
  filler sequence-5
SGGSG

SEQ ID NO: 6 - protein, 5 aa, Artificial Sequence
  filler sequence-6
GGGGS

SEQ ID NO: 7 - protein, 6 aa, Artificial Sequence
  filler sequence-7
GGSGGS

SEQ ID NO: 8 - protein, 7 aa, Artificial Sequence
  filler sequence-8
GGSGGSG

SEQ ID NO: 9 - protein, 8 aa, Artificial Sequence
  filler sequence-9
SGSGGSGS

SEQ ID NO: 10 - protein, 9 aa, Artificial Sequence
  filler sequence-10
GSGGSGSGS

SEQ ID NO: 11 - protein, 10 aa, Artificial Sequence
  filler sequence-11
SGGSGGSGSG

SEQ ID NO: 12 - protein, 11 aa, Artificial Sequence
  filler sequence-12
GGSGGSGGSGS

SEQ ID NO: 13 - protein, 12 aa, Artificial Sequence
  filler sequence-13
SGGSGGSGSGGS

SEQ ID NO: 14 - protein, 13 aa, Artificial Sequence
  filler sequence-14
GGGGSGGSGGGGS

SEQ ID NO: 15 - protein, 14 aa, Artificial Sequence
  filler sequence-15
GGGSGSGSGSGGGS

SEQ ID NO: 16 - protein, 15 aa, Artificial Sequence
  filler sequence-16
SGSGGGGGSGGSGSG

SEQ ID NO: 17 - protein, 16 aa, Artificial Sequence
  MOD_RES 1: ACETYLATION
  polypeptide core
CGGSGGSGGSKGSGSK

SEQ ID NO: 18 - protein, 19 aa, Artificial Sequence
  MOD_RES 1: ACETYLATION
  polypeptitde core-1
CGGSGGSGGSKGSGSKGSK

SEQ ID NO: 19 - protein, 31 aa, Artificial Sequence
  MOD_RES 1: ACETYLATION
  polypeptide core
CGSKGSKGSKGSKGSKGSKGSKGSKGSKGSK

SEQ ID NO: 20 - protein, 16 aa, Artificial Sequence
  MOD_RES 1: Xaa is homopropargylglycine
  MOD_RES 1: ACETYLATION
  polypeptide core
XGGSGGSGGSKGSGSK

SEQ ID NO: 21 - protein, 19 aa, Artificial Sequence
  MOD_RES 1: Xaa is homopropargylglycine
  MOD_RES 1: ACETYLATION
  polypeptide core
XGGSGGSGGSKGSGSKGSK

SEQ ID NO: 22 - protein, 19 aa, Artificial Sequence
  MOD_RES 1: Xaa is L-azidohomoalanine
  MOD_RES 1: ACETYLATION
  polypeptide core
XGGSGGSGGSKGSGSKGSK

SEQ ID NO: 23 - protein, 21 aa, Artificial Sequence
  MOD_RES 1: Xaa is homopropargylglycine
  MOD_RES 1: ACETYLATION
  polypeptide core
XGGSGGSGGSKGSGSKGSGSC

SEQ ID NO: 24 - protein, 7 aa, Artificial Sequence
  MOD_RES 1: ACETYLATION
  polypeptide core
  MOD_RES 2,4,6: Xaa is PEGylated amino acid with two EG units
CXKXKXK

SEQ ID NO: 25 - protein, 11 aa, Artificial Sequence
  MOD_RES 1: ACETYLATION
  polypeptide core
  MOD_RES 2,4,6,8,10: Xaa is PEGylated amino acid with six EG units
CXKXKXKXKXK

SEQ ID NO: 26 - protein, 16 aa, Artificial Sequence
  polypeptide core-2
CGSKGSKGSKGSKGSK

SEQ ID NO: 27 - protein, 250 aa, Artificial Sequence
  anti-fibrin scFv 102-10
DIQMTQSPSSLSASLGGKVTITCKASQDINKYIAWFQHKPGKGPRLLIHYTSTLQPGIPSRFSGSGSGRDYSFSISNLEPEDLATYYCLQYDNLTWTFGGGTKLEIKRGSTSGSGKPGSGEGSTKGQIQLVQSGPELKKPGETVKISCKASGYTFTNYGMNWVKQAPGKGLKWMGWINTYTGEATYADDFKGRFAFSLETSANTAYVQINNLKNEDTATYFCARLMDYWGQGTSVTVSSGGGGSGGGGSC

SEQ ID NO: 28 - protein, 366 aa, Artificial Sequence
  reteplase-Cys
SYQGNSDCYFGNGSAYRGTHSLTESGASCLPWNSMILIGKVYTAQNPSAQALGLGKHNYCRNPDGDAKPWCHVLKNRRLTWEYCDVPSCSTCGLRQYSQPQFRIKGGLFADIASHPWQAAIFAKHRRSPGERFLCGGILISSCWILSAAHCFQERFPPHHLTVILGRTYRVVPGEEEQKFEVEKYIVHKEFDDDTYDNDIALLQLKSDSSRCAQESSVVRTVCLPPADLQLPDWTECELSGYGKHEALSPFYSERLKEAHVRLYPSSRCTSQHLLNRTVTDNMLCAGDTRSGGPQANLHDACQGDSGGPLVCLNDGRMTLVGIISWGLGCGQKDVPGVYTKVTNYLDWIRDNMRPGGGGSGGGGSC

SEQ ID NO: 29 - protein, 244 aa, Artificial Sequence
  Phage-displayed anti-fibrin scFv D10
DIQMTQSPSSLSASVGDRVTITCRASQDVGFYVAWYQQKPGKAPKLLISYPSGLYSGVPSRFSGSGSGTDFTLTISSLQPEDFATYYCQQYYDYPITFGQGTKVEIKRGSTSGSGKPGSGEGSTKGEVQLVESGGGLVQPGGSLRLSCAASGFTINDFSIHWVRQAPGKGLEWVAGIWPYGGYTFYADSVKGRFTISADTSKNTAYLRMNSLRAEDTAVYYCARFGYYSFGDYWGQGTLVTVSS

SEQ ID NO: 30 - protein, 599 aa, Artificial Sequence
  2-chain IgG4.Fc fusion protein containing reteplase
SYQGNSDCYFGNGSAYRGTHSLTESGASCLPWNSMILIGKVYTAQNPSAQALGLGKHNYCRNPDGDAKPWCHVLKNRRLTWEYCDVPSCSTCGLRQYSQPQFRIKGGLFADIASHPWQAAIFAKHRRSPGERFLCGGILISSCWILSAAHCFQERFPPHHLTVILGRTYRVVPGEEEQKFEVEKYIVHKEFDDDTYDNDIALLQLKSDSSRCAQESSVVRTVCLPPADLQLPDWTECELSGYGKHEALSPFYSERLKEAHVRLYPSSRCTSQHLLNRTVTDNMLCAGDTRSGGPQANLHDACQGDSGGPLVCLNDGRMTLVGIISWGLGCGQKDVPGVYTKVTNYLDWIRDNMRPASGGSPPCPSCPAPEFLGGPSVFLFPPKPKDTLMISRTPEVTCVVVDVSQEDPEVQFNWYVDGVEVHNAKTKPREEQFNSTYRVVSVLTVLHQDWLNGKEYKCKVSNKGLPSSIEKTISKAKGQPREPQVYTLPPSQEEMTKNQVSLTCLVKGFYPSDIAVEWESNGQPENNYKTTPPVLDSDGSFFLYSRLTVDKSRWQEGNVFSCSVMHEALHNHYTQKSLSLSLGKGGGGSGGGGSGGGGS

SEQ ID NO: 31 - protein, 838 aa, Artificial Sequence
  (reteplase)-hIgG4.Fc-(scFv α fibrin 102-10)
SYQGNSDCYFGNGSAYRGTHSLTESGASCLPWNSMILIGKVYTAQNPSAQALGLGKHNYCRNPDGDAKPWCHVLKNRRLTWEYCDVPSCSTCGLRQYSQPQFRIKGGLFADIASHPWQAAIFAKHRRSPGERFLCGGILISSCWILSAAHCFQERFPPHHLTVILGRTYRVVPGEEEQKFEVEKYIVHKEFDDDTYDNDIALLQLKSDSSRCAQESSVVRTVCLPPADLQLPDWTECELSGYGKHEALSPFYSERLKEAHVRLYPSSRCTSQHLLNRTVTDNMLCAGDTRSGGPQANLHDACQGDSGGPLVCLNDGRMTLVGIISWGLGCGQKDVPGVYTKVTNYLDWIRDNMRPASGGSPPCPSCPAPEFLGGPSVFLFPPKPKDTLMISRTPEVTCVVVDVSQEDPEVQFNWYVDGVEVHNAKTKPREEQFNSTYRVVSVLTVLHQDWLNGKEYKCKVSNKGLPSSIEKTISKAKGQPREPQVYTLPPSQEEMTKNQVSLTCLVKGFYPSDIAVEWESNGQPENNYKTTPPVLDSDGSFFLYSRLTVDKSRWQEGNVFSCSVMHEALHNHYTQKSLSLSLGKGGGGSGGGGSGGGGSDIQMTQSPSSLSASLGGKVTITCKASQDINKYIAWFQHKPGKGPRLLIHYTSTLQPGIPSRFSGSGSGRDYSFSISNLEPEDLATYYCLQYDNLTWTFGGGTKLEIKRGSTSGSGKPGSGEGSTKGQIQLVQSGPELKKPGETVKISCKASGYTFTNYGMNWVKQAPGKGLKWMGWINTYTGEATYADDFKGRFAFSLETSANTAYVQINNLKNEDTATYFCARLMDYWGQGTSVTVSS

SEQ ID NO: 32 - protein, 611 aa, Artificial Sequence
  (reteplase)-(scFv α fibrin 102-10)
SYQGNSDCYFGNGSAYRGTHSLTESGASCLPWNSMILIGKVYTAQNPSAQALGLGKHNYCRNPDGDAKPWCHVLKNRRLTWEYCDVPSCSTCGLRQYSQPQFRIKGGLFADIASHPWQAAIFAKHRRSPGERFLCGGILISSCWILSAAHCFQERFPPHHLTVILGRTYRVVPGEEEQKFEVEKYIVHKEFDDDTYDNDIALLQLKSDSSRCAQESSVVRTVCLPPADLQLPDWTECELSGYGKHEALSPFYSERLKEAHVRLYPSSRCTSQHLLNRTVTDNMLCAGDTRSGGPQANLHDACQGDSGGPLVCLNDGRMTLVGIISWGLGCGQKDVPGVYTKVTNYLDWIRDNMRPASGGGGSGGGGSGGGGSDIQMTQSPSSLSASLGGKVTITCKASQDINKYIAWFQHKPGKGPRLLIHYTSTLQPGIPSRFSGSGSGRDYSFSISNLEPEDLATYYCLQYDNLTWTFGGGTKLEIKRGSTSGSGKPGSGEGSTKGQIQLVQSGPELKKPGETVKISCKASGYTFTNYGMNWVKQAPGKGLKWMGWINTYTGEATYADDFKGRFAFSLETSANTAYVQINNLKNEDTATYFCARLMDYWGQGTSVTVSS

SEQ ID NO: 33 - protein, 771 aa, Artificial Sequence
  2-chain IgG4.Fc fusion protein containing TNK-tPA
SYQVICRDEKTQMIYQQHQSWLRPVLRSNRVEYCWCNSGRAQCHSVPVKSCSEPRCFNGGTCQQALYFSDFVCQCPEGFAGKCCEIDTRATCYEDQGISYRGNWSTAESGAECTQWNSSALAQKPYSGRRPDAIRLGLGNHNYCRNPDRDSKPWCYVFKAGKYSSEFCSTPACSEGNSDCYFGNGSAYRGTHSLTESGASCLPWNSMILIGKVYTAQNPSAQALGLGKHNYCRNPDGDAKPWCHVLKNRRLTWEYCDVPSCSTCGLRQYSQPQFRIKGGLFADIASHPWQAAAAAKHRRSPGERFLCGGILISSCWILSAAHCFQERFPPHHLTVILGRTYRVVPGEEEQKFEVEKYIVHKEFDDDTYDNDIALLQLKSDSSRCAQESSVVRTVCLPPADLQLPDWTECELSGYGKHEALSPFYSERLKEAHVRLYPSSRCTSQHLLNRTVTDNMLCAGDTRSGGPQANLHDACQGDSGGPLVCLNDGRMTLVGIISWGLGCGQKDVPGVYTKVTNYLDWIRDNMRPASGGSPPCPSCPAPEFLGGPSVFLFPPKPKDTLMISRTPEVTCVVVDVSQEDPEVQFNWYVDGVEVHNAKTKPREEQFNSTYRVVSVLTVLHQDWLNGKEYKCKVSNKGLPSSIEKTISKAKGQPREPQVYTLPPSQEEMTKNQVSLTCLVKGFYPSDIAVEWESNGQPENNYKTTPPVLDSDGSFFLYSRLTVDKSRWQEGNVFSCSVMHEALHNHYTQKSLSLSLGKGGGGSGGGGSGGGGS

SEQ ID NO: 34 - protein, 1015 aa, Artificial Sequence
  (TNK-tPA)-hIgG4.Fc-(scFv α fibrin D10)
SYQVICRDEKTQMIYQQHQSWLRPVLRSNRVEYCWCNSGRAQCHSVPVKSCSEPRCFNGGTCQQALYFSDFVCQCPEGFAGKCCEIDTRATCYEDQGISYRGNWSTAESGAECTQWNSSALAQKPYSGRRPDAIRLGLGNHNYCRNPDRDSKPWCYVFKAGKYSSEFCSTPACSEGNSDCYFGNGSAYRGTHSLTESGASCLPWNSMILIGKVYTAQNPSAQALGLGKHNYCRNPDGDAKPWCHVLKNRRLTWEYCDVPSCSTCGLRQYSQPQFRIKGGLFADIASHPWQAAAAAKHRRSPGERFLCGGILISSCWILSAAHCFQERFPPHHLTVILGRTYRVVPGEEEQKFEVEKYIVHKEFDDDTYDNDIALLQLKSDSSRCAQESSVVRTVCLPPADLQLPDWTECELSGYGKHEALSPFYSERLKEAHVRLYPSSRCTSQHLLNRTVTDNMLCAGDTRSGGPQANLHDACQGDSGGPLVCLNDGRMTLVGIISWGLGCGQKDVPGVYTKVTNYLDWIRDNMRPASGGSPPCPSCPAPEFLGGPSVFLFPPKPKDTLMISRTPEVTCVVVDVSQEDPEVQFNWYVDGVEVHNAKTKPREEQFNSTYRVVSVLTVLHQDWLNGKEYKCKVSNKGLPSSIEKTISKAKGQPREPQVYTLPPSQEEMTKNQVSLTCLVKGFYPSDIAVEWESNGQPENNYKTTPPVLDSDGSFFLYSRLTVDKSRWQEGNVFSCSVMHEALHNHYTQKSLSLSLGKGGGGSGGGGSGGGGSDIQMTQSPSSLSASVGDRVTITCRASQDVGFYVAWYQQKPGKAPKLLISYPSGLYSGVPSRFSGSGSGTDFTLTISSLQPEDFATYYCQQYYDYPITFGQGTKVEIKRGSTSGSGKPGSGEGSTKGEVQLVESGGGLVQPGGSLRLSCAASGFTINDFSIHWVRQAPGKGLEWVAGIWPYGGYTFYADSVKGRFTISADTSKNTAYLRMNSLRAEDTAVYYCARFGYYSFGDYWGQGTLVTVSS

SEQ ID NO: 35 - protein, 788 aa, Artificial Sequence
  (TNK-tPA)-(scFv α fibrin)
SYQVICRDEKTQMIYQQHQSWLRPVLRSNRVEYCWCNSGRAQCHSVPVKSCSEPRCFNGGTCQQALYFSDFVCQCPEGFAGKCCEIDTRATCYEDQGISYRGNWSTAESGAECTQWNSSALAQKPYSGRRPDAIRLGLGNHNYCRNPDRDSKPWCYVFKAGKYSSEFCSTPACSEGNSDCYFGNGSAYRGTHSLTESGASCLPWNSMILIGKVYTAQNPSAQALGLGKHNYCRNPDGDAKPWCHVLKNRRLTWEYCDVPSCSTCGLRQYSQPQFRIKGGLFADIASHPWQAAAAAKHRRSPGERFLCGGILISSCWILSAAHCFQERFPPHHLTVILGRTYRVVPGEEEQKFEVEKYIVHKEFDDDTYDNDIALLQLKSDSSRCAQESSVVRTVCLPPADLQLPDWTECELSGYGKHEALSPFYSERLKEAHVRLYPSSRCTSQHLLNRTVTDNMLCAGDTRSGGPQANLHDACQGDSGGPLVCLNDGRMTLVGIISWGLGCGQKDVPGVYTKVTNYLDWIRDNMRPASGGGGSGGGGSGGGGSDIQMTQSPSSLSASVGDRVTITCRASQDVGFYVAWYQQKPGKAPKLLISYPSGLYSGVPSRFSGSGSGTDFTLTISSLQPEDFATYYCQQYYDYPITFGQGTKVEIKRGSTSGSGKPGSGEGSTKGEVQLVESGGGLVQPGGSLRLSCAASGFTINDFSIHWVRQAPGKGLEWVAGIWPYGGYTFYADSVKGRFTISADTSKNTAYLRMNSLRAEDTAVYYCARFGYYSFGDYWGQGTLVTVSS